European Patent Specification EP 3 741 381 B1, published April 24, 2024. Title: METHODS FOR PREVENTION AND TREATMENT OF ACUTE RENAL INJURY. Applicant: CORNELL UNIVERSITY. Application PCT/US2009/35132. The sequence listing filed with the application follows.

SEQUENCE LISTING (2 sequences)

SEQ ID NO: 1 - DNA, 20 bp, Artificial Sequence
  Description of Artificial Sequence: Synthetic primer
ctgaagaagattgcgcagaa

SEQ ID NO: 2 - DNA, 20 bp, Artificial Sequence
  Description of Artificial Sequence: Synthetic primer
atggcataaattcccactgc